European Patent Specification EP 3 683 235 B1, published May 22, 2024. Title: Anti-IL-33 Antibodies and Uses Thereof. Applicant: Regeneron Pharmaceuticals, Inc. Application TBA. The sequence listing filed with the application follows.

SEQUENCE LISTING (323 sequences)

SEQ ID NO: 1 - DNA, 366 bp, Artificial Sequence
  Synthetic
caggtgcagctggtggagtctgggggaggcgtggtccagcctgggaggtccctgagactctcctgtgcagcgtctggattcaccttcagtagttatggcatgcattgggtccgccaggctccaggcaaggggctggagtgggtggcagttatatggtatgatggaagaaataaatactatacagactccgtgaagggccgattcaccatctccagagacaattccaagaacacgctgtatctgcaaatggacagcctgagagccgaggacacggctgtgtattactgtgcgagagagaggtatatcagcagctattatggggggttcgacccctggggccagggagccctggtcaccgtctcctca

SEQ ID NO: 2 - protein, 122 aa, Artificial Sequence
  Synthetic
QVQLVESGGGVVQPGRSLRLSCAASGFTFSSYGMHWVRQAPGKGLEWVAVIWYDGRNKYYTDSVKGRFTISRDNSKNTLYLQMDSLRAEDTAVYYCARERYISSYYGGFDPWGQGALVTVSS

SEQ ID NO: 3 - DNA, 24 bp, Artificial Sequence
  Synthetic
ggattcaccttcagtagttatggc

SEQ ID NO: 4 - protein, 8 aa, Artificial Sequence
  Synthetic
GFTFSSYG

SEQ ID NO: 5 - DNA, 24 bp, Artificial Sequence
  Synthetic
atatggtatgatggaagaaataaa

SEQ ID NO: 6 - protein, 8 aa, Artificial Sequence
  Synthetic
IWYDGRNK

SEQ ID NO: 7 - DNA, 45 bp, Artificial Sequence
  Synthetic
gcgagagagaggtatatcagcagctattatggggggttcgacccc

SEQ ID NO: 8 - protein, 15 aa, Artificial Sequence
  Synthetic
ARERYISSYYGGFDP

SEQ ID NO: 9 - DNA, 321 bp, Artificial Sequence
  Synthetic
gacatccagatgacccagtctccatcctccgtgtctgcatctgtaggagacagagtcaccatcacttgtcgggcgagtcagggtattagtagttggttagcctggtatcagcagaaaccagggaaagcccctaaggtcctgatctatgctgcatccagtttgcaaagtggggtcccatcaaggttcagcggcagtggatctgggacagatttcactctcaccatcagcagcctgcagcctgaagattttgcaacttactattgtcaacaggctaacagtttcccattcactttcggccctgggaccaaactggatatcaag

SEQ ID NO: 10 - protein, 107 aa, Artificial Sequence
  Synthetic
DIQMTQSPSSVSASVGDRVTITCRASQGISSWLAWYQQKPGKAPKVLIYAASSLQSGVPSRFSGSGSGTDFTLTISSLQPEDFATYYCQQANSFPFTFGPGTKLDIK

SEQ ID NO: 11 - DNA, 18 bp, Artificial Sequence
  Synthetic
cagggtattagtagttgg

SEQ ID NO: 12 - protein, 6 aa, Artificial Sequence
  Synthetic
QGISSW

SEQ ID NO: 13 - DNA, 9 bp, Artificial Sequence
  Synthetic
gctgcatcc

SEQ ID NO: 14 - protein, 3 aa, Artificial Sequence
  Synthetic
AAS

SEQ ID NO: 15 - DNA, 27 bp, Artificial Sequence
  Synthetic
caacaggctaacagtttcccattcact

SEQ ID NO: 16 - protein, 9 aa, Artificial Sequence
  Synthetic
QQANSFPFT

SEQ ID NO: 17 - DNA, 357 bp, Artificial Sequence
  Synthetic
gaggtgcagctgttggagtctgggggagacttggtacagcctggggggtccctgagactctcctgtgcagcctctggattcaccttcagcagctatgccatgagctgggtccgccaggctccagggaaggggctggagtgggtctcagttattagtggtagtggaagtagcacagactacgcagactccgtgaagggccggttcaccatttccagagacaattccagggacacgctgcatctgcaaatgaacagcctgagagccgaggacacggccgtatattactgtgcgaaaacgttctactacttctacggtttggacgtctggggccaagggaccacggtcaccgtctcctca

SEQ ID NO: 18 - protein, 119 aa, Artificial Sequence
  Synthetic
EVQLLESGGDLVQPGGSLRLSCAASGFTFSSYAMSWVRQAPGKGLEWVSVISGSGSSTDYADSVKGRFTISRDNSRDTLHLQMNSLRAEDTAVYYCAKTFYYFYGLDVWGQGTTVTVSS

SEQ ID NO: 19 - DNA, 24 bp, Artificial Sequence
  Synthetic
ggattcaccttcagcagctatgcc

SEQ ID NO: 20 - protein, 8 aa, Artificial Sequence
  Synthetic
GFTFSSYA

SEQ ID NO: 21 - DNA, 24 bp, Artificial Sequence
  Synthetic
attagtggtagtggaagtagcaca

SEQ ID NO: 22 - protein, 8 aa, Artificial Sequence
  Synthetic
ISGSGSST

SEQ ID NO: 23 - DNA, 36 bp, Artificial Sequence
  Synthetic
gcgaaaacgttctactacttctacggtttggacgtc

SEQ ID NO: 24 - protein, 12 aa, Artificial Sequence
  Synthetic
AKTFYYFYGLDV

SEQ ID NO: 25 - DNA, 321 bp, Artificial Sequence
  Synthetic
gacatccagatgacccagtctccatcctccctgtctgcatctttaagagacagagtcaccatcacttgccgggcgagtcagggcattagcaattatttagcctggtatcagcagaaaccagggaaagttcctaaggtcctaatctatgctgcatccactttgcaatcaggggtcccatctcggttcagtggcagtggatctgggacagttttcactctcaccatcagcagcctgcagactgaagatgttgcaacttattactgtcaaaagtatagcagtgccccattcactttcggccctgggaccaaagtggatatcaaa

SEQ ID NO: 26 - protein, 107 aa, Artificial Sequence
  Synthetic
DIQMTQSPSSLSASLRDRVTITCRASQGISNYLAWYQQKPGKVPKVLIYAASTLQSGVPSRFSGSGSGTVFTLTISSLQTEDVATYYCQKYSSAPFTFGPGTKVDIK

SEQ ID NO: 27 - DNA, 18 bp, Artificial Sequence
  Synthetic
cagggcattagcaattat

SEQ ID NO: 28 - protein, 6 aa, Artificial Sequence
  Synthetic
QGISNY

SEQ ID NO: 29 - DNA, 9 bp, Artificial Sequence
  Synthetic
gctgcatcc

SEQ ID NO: 30 - protein, 3 aa, Artificial Sequence
  Synthetic
AAS

SEQ ID NO: 31 - DNA, 27 bp, Artificial Sequence
  Synthetic
caaaagtatagcagtgccccattcact

SEQ ID NO: 32 - protein, 9 aa, Artificial Sequence
  Synthetic
QKYSSAPFT

SEQ ID NO: 33 - DNA, 351 bp, Artificial Sequence
  Synthetic
caggtgcttctggtacagtctggggctgaggtgaagaagcctggggccacagtgaaggtctcctgcaaggcttctggatccactttcaccggctactatatgcactgggtgcgacaggcccctggacaagggcttgagtggatgggatggatcaaccctaacaatggtggcacaaactatgcacagaagtttcagggcagggtcaccatgaccagggacacgtccatcagcacagcctacatggaattgagcaggctgagatctgacgacacggccgtatattactgtgcgagagagttgcggtataactggaagtcctggggccagggaaccctggtcaccgtctcctca

SEQ ID NO: 34 - protein, 117 aa, Artificial Sequence
  Synthetic
QVLLVQSGAEVKKPGATVKVSCKASGSTFTGYYMHWVRQAPGQGLEWMGWINPNNGGTNYAQKFQGRVTMTRDTSISTAYMELSRLRSDDTAVYYCARELRYNWKSWGQGTLVTVSS

SEQ ID NO: 35 - DNA, 24 bp, Artificial Sequence
  Synthetic
ggatccactttcaccggctactat

SEQ ID NO: 36 - protein, 8 aa, Artificial Sequence
  Synthetic
GSTFTGYY

SEQ ID NO: 37 - DNA, 24 bp, Artificial Sequence
  Synthetic
atcaaccctaacaatggtggcaca

SEQ ID NO: 38 - protein, 8 aa, Artificial Sequence
  Synthetic
INPNNGGT

SEQ ID NO: 39 - DNA, 30 bp, Artificial Sequence
  Synthetic
gcgagagagttgcggtataactggaagtcc

SEQ ID NO: 40 - protein, 10 aa, Artificial Sequence
  Synthetic
ARELRYNWKS

SEQ ID NO: 41 - DNA, 324 bp, Artificial Sequence
  Synthetic
gaaattgtgttgacgcagtctccaggcaccctgtctttgtctccaggggaaagagtcaccctctcctgcagggccagtcagagtgttggcaggccctacttagcctggtaccaacagatacctggccaggctcccaggctcctcatctatggtgcatccagcagggccactgacatcccagacaggttcagtggcaatgggtctgggacagacttcactctcaccatcagtagactggagcctgaagattttgcagtgtattactgtcagcagtatgataattccccttatacttttggccaggggaccaggctggagatcaaa

SEQ ID NO: 42 - protein, 108 aa, Artificial Sequence
  Synthetic
EIVLTQSPGTLSLSPGERVTLSCRASQSVGRPYLAWYQQIPGQAPRLLIYGASSRATDIPDRFSGNGSGTDFTLTISRLEPEDFAVYYCQQYDNSPYTFGQGTRLEIK

SEQ ID NO: 43 - DNA, 21 bp, Artificial Sequence
  Synthetic
cagagtgttggcaggccctac

SEQ ID NO: 44 - protein, 7 aa, Artificial Sequence
  Synthetic
QSVGRPY

SEQ ID NO: 45 - DNA, 9 bp, Artificial Sequence
  Synthetic
ggtgcatcc

SEQ ID NO: 46 - protein, 3 aa, Artificial Sequence
  Synthetic
GAS

SEQ ID NO: 47 - DNA, 27 bp, Artificial Sequence
  Synthetic
cagcagtatgataattccccttatact

SEQ ID NO: 48 - protein, 9 aa, Artificial Sequence
  Synthetic
QQYDNSPYT

SEQ ID NO: 49 - DNA, 366 bp, Artificial Sequence
  Synthetic
gaggtgcagctggtggagtctgggggaggcttggtacaacctggggggtccctgagactctcctgtgcagcctctggattcacctttagaagctttgccatgagctgggtccgccaggctccagggaaggggctggaattggtctcagatctcaggactagtggtggtagtacatactacgcagactccgtgaagggccggctcaccatctccagagacaattccaagaacacgctgtatctgcaaatgaacagcctgagagccgaggacacggccgtatattactgtgcgaaaagccactatagcaccagctggttcgggggctttgactactggggccagggaaccctggtcactgtctcctca

SEQ ID NO: 50 - protein, 122 aa, Artificial Sequence
  Synthetic
EVQLVESGGGLVQPGGSLRLSCAASGFTFRSFAMSWVRQAPGKGLELVSDLRTSGGSTYYADSVKGRLTISRDNSKNTLYLQMNSLRAEDTAVYYCAKSHYSTSWFGGFDYWGQGTLVTVSS

SEQ ID NO: 51 - DNA, 24 bp, Artificial Sequence
  Synthetic
ggattcacctttagaagctttgcc

SEQ ID NO: 52 - protein, 8 aa, Artificial Sequence
  Synthetic
GFTFRSFA

SEQ ID NO: 53 - DNA, 24 bp, Artificial Sequence
  Synthetic
ctcaggactagtggtggtagtaca

SEQ ID NO: 54 - protein, 8 aa, Artificial Sequence
  Synthetic
LRTSGGST

SEQ ID NO: 55 - DNA, 45 bp, Artificial Sequence
  Synthetic
gcgaaaagccactatagcaccagctggttcgggggctttgactac

SEQ ID NO: 56 - protein, 15 aa, Artificial Sequence
  Synthetic
AKSHYSTSWFGGFDY

SEQ ID NO: 57 - DNA, 321 bp, Artificial Sequence
  Synthetic
gacatccagatgacccagtctccatcttccgtgtctgcttctgtaggagacagagtcaccatcacttgtcgggcgagtcagggttttagcagctggttagcctggtatcagcagaaaccagggaaagcccctaagctcctgatctatgctgcatccagtttgcaaagtggggtcccatcaaggttcagcggcagtggatctgggacagatttcactctcaccatcaccaacctgcagcctgaagattttgcaacttactattgtcaacaggctaacagtttccctctcactttcggcggagggaccaaggtggagatcaaa

SEQ ID NO: 58 - protein, 107 aa, Artificial Sequence
  Synthetic
DIQMTQSPSSVSASVGDRVTITCRASQGFSSWLAWYQQKPGKAPKLLIYAASSLQSGVPSRFSGSGSGTDFTLTITNLQPEDFATYYCQQANSFPLTFGGGTKVEIK

SEQ ID NO: 59 - DNA, 18 bp, Artificial Sequence
  Synthetic
cagggttttagcagctgg

SEQ ID NO: 60 - protein, 6 aa, Artificial Sequence
  Synthetic
QGFSSW

SEQ ID NO: 61 - DNA, 9 bp, Artificial Sequence
  Synthetic
gctgcatcc

SEQ ID NO: 62 - protein, 3 aa, Artificial Sequence
  Synthetic
AAS

SEQ ID NO: 63 - DNA, 27 bp, Artificial Sequence
  Synthetic
caacaggctaacagtttccctctcact

SEQ ID NO: 64 - protein, 9 aa, Artificial Sequence
  Synthetic
QQANSFPLT

SEQ ID NO: 65 - DNA, 366 bp, Artificial Sequence
  Synthetic
gaggtgcagctggtggagtctgggggaggcttggtacagcctggggggtccctgagactctcctgtgcagcctctggattcacgtttagcagctatgtcatgagctgggtccgccaggctccagggaaggggctggagtgggtctcaagtattagtggtaatggtggtagcacaaactacgcagactccgtgaagggccggttcaccatctccagagacaattccaagaacacgctgtttctggaaatgaacagcctgagagccgaggacacggccgtatattactgtgcgaaatcactgggaactaccacgacttttttggggtttgactattggggccagggaaccctggtcaccgtctcctca

SEQ ID NO: 66 - protein, 122 aa, Artificial Sequence
  Synthetic
EVQLVESGGGLVQPGGSLRLSCAASGFTFSSYVMSWVRQAPGKGLEWVSSISGNGGSTNYADSVKGRFTISRDNSKNTLFLEMNSLRAEDTAVYYCAKSLGTTTTFLGFDYWGQGTLVTVSS

SEQ ID NO: 67 - DNA, 24 bp, Artificial Sequence
  Synthetic
ggattcacgtttagcagctatgtc

SEQ ID NO: 68 - protein, 8 aa, Artificial Sequence
  Synthetic
GFTFSSYV

SEQ ID NO: 69 - DNA, 24 bp, Artificial Sequence
  Synthetic
attagtggtaatggtggtagcaca

SEQ ID NO: 70 - protein, 8 aa, Artificial Sequence
  Synthetic
ISGNGGST

SEQ ID NO: 71 - DNA, 45 bp, Artificial Sequence
  Synthetic
gcgaaatcactgggaactaccacgacttttttggggtttgactat

SEQ ID NO: 72 - protein, 15 aa, Artificial Sequence
  Synthetic
AKSLGTTTTFLGFDY

SEQ ID NO: 73 - DNA, 321 bp, Artificial Sequence
  Synthetic
gacatccagatgacccagtctccatcttccgtgtctgcatctgtaggagacagagtcaccatcacttgtcgggcgagtcagggtattagcagctggttagcctggtatcagcagaaaccagggaaagcccctaaactcctgatctatgctgcatccagtttgcaaagtggggtcccatcaaggttcagcggcagtggatctgggacatatttcactctcaccatcagcagcctgcagcctgaagattttgcaacttactattgtcaacaggctaacagtttccctctcactttcggcggagggaccaaggtggagatcaaa

SEQ ID NO: 74 - protein, 107 aa, Artificial Sequence
  Synthetic
DIQMTQSPSSVSASVGDRVTITCRASQGISSWLAWYQQKPGKAPKLLIYAASSLQSGVPSRFSGSGSGTYFTLTISSLQPEDFATYYCQQANSFPLTFGGGTKVEIK

SEQ ID NO: 75 - DNA, 18 bp, Artificial Sequence
  Synthetic
cagggtattagcagctgg

SEQ ID NO: 76 - protein, 6 aa, Artificial Sequence
  Synthetic
QGISSW

SEQ ID NO: 77 - DNA, 9 bp, Artificial Sequence
  Synthetic
gctgcatcc

SEQ ID NO: 78 - protein, 3 aa, Artificial Sequence
  Synthetic
AAS

SEQ ID NO: 79 - DNA, 27 bp, Artificial Sequence
  Synthetic
caacaggctaacagtttccctctcact

SEQ ID NO: 80 - protein, 9 aa, Artificial Sequence
  Synthetic
QQANSFPLT

SEQ ID NO: 81 - DNA, 363 bp, Artificial Sequence
  Synthetic
caggtgcagctgcaggagtcgggcccaggactggtgaagccttcggagaccctgtccctcacctgcactgtctctggtggctccatcagtagttattactggagctggatccggcagcccccagggaagggactggagttgattgggtatatttattacagtgggagcaccaattataacccctccctcaagagtcgagtcaccatatctgtagacacgtccaagaaccacttctccctgaagctgagctctgtgaccgctgcggacacggccgtatattactgtgcgagatcccagtataccagtagttggtacggttcttttgatatctggggccaagggacaatggtcaccgtctcttca

SEQ ID NO: 82 - protein, 121 aa, Artificial Sequence
  Synthetic
QVQLQESGPGLVKPSETLSLTCTVSGGSISSYYWSWIRQPPGKGLELIGYIYYSGSTNYNPSLKSRVTISVDTSKNHFSLKLSSVTAADTAVYYCARSQYTSSWYGSFDIWGQGTMVTVSS

SEQ ID NO: 83 - DNA, 24 bp, Artificial Sequence
  Synthetic
ggtggctccatcagtagttattac

SEQ ID NO: 84 - protein, 8 aa, Artificial Sequence
  Synthetic
GGSISSYY

SEQ ID NO: 85 - DNA, 21 bp, Artificial Sequence
  Synthetic
atttattacagtgggagcacc

SEQ ID NO: 86 - protein, 7 aa, Artificial Sequence
  Synthetic
IYYSGST

SEQ ID NO: 87 - DNA, 45 bp, Artificial Sequence
  Synthetic
gcgagatcccagtataccagtagttggtacggttcttttgatatc

SEQ ID NO: 88 - protein, 15 aa, Artificial Sequence
  Synthetic
ARSQYTSSWYGSFDI

SEQ ID NO: 89 - DNA, 321 bp, Artificial Sequence
  Synthetic
gacatccagatgacccagtctccatcttccgtgtctgcatctgtaggagacagagtcaccatcacttgtcgggcgagtcagggtattagcacctggttagcctggtttcagcagaaaccagggaaagcccctaagctcctgatctatgctgcatccactttacaaggtggggtcccatcaaggttcagcggcagtggatctgggccagaattcactctcaccatcagcagcctgcagcctgaagattttgcaacttactattgtcaacaggctaacagtttcccgtggacgttcggccaagggaccaaggtggaaatcaaa

SEQ ID NO: 90 - protein, 107 aa, Artificial Sequence
  Synthetic
DIQMTQSPSSVSASVGDRVTITCRASQGISTWLAWFQQKPGKAPKLLIYAASTLQGGVPSRFSGSGSGPEFTLTISSLQPEDFATYYCQQANSFPWTFGQGTKVEIK

SEQ ID NO: 91 - DNA, 18 bp, Artificial Sequence
  Synthetic
cagggtattagcacctgg

SEQ ID NO: 92 - protein, 6 aa, Artificial Sequence
  Synthetic
QGISTW

SEQ ID NO: 93 - DNA, 9 bp, Artificial Sequence
  Synthetic
gctgcatcc

SEQ ID NO: 94 - protein, 3 aa, Artificial Sequence
  Synthetic
AAS

SEQ ID NO: 95 - DNA, 27 bp, Artificial Sequence
  Synthetic
caacaggctaacagtttcccgtggacg

SEQ ID NO: 96 - protein, 9 aa, Artificial Sequence
  Synthetic
QQANSFPWT

SEQ ID NO: 97 - DNA, 366 bp, Artificial Sequence
  Synthetic
caggttcagctggtgcagtctggagctgaggtgaagaagcctggggcctcagtgaaggtctcctgcaaggcctctggttacacctttaacagctatggtatcagctgggtgcgacaggcccctggacaagggcttgagtggatgggatggatcagctcccacaatggtaacagtcactatgtacagaagttccagggcagagtctccatgaccacagacacatccacgagtacagcctacatggaactgaggagccttagatctgacgacacggccgtgtattactgtgcgagacactcgtataccaccagctggtacgggggttttgactattggggccagggaaccctggtcaccgtctcctca

SEQ ID NO: 98 - protein, 122 aa, Artificial Sequence
  Synthetic
QVQLVQSGAEVKKPGASVKVSCKASGYTFNSYGISWVRQAPGQGLEWMGWISSHNGNSHYVQKFQGRVSMTTDTSTSTAYMELRSLRSDDTAVYYCARHSYTTSWYGGFDYWGQGTLVTVSS

SEQ ID NO: 99 - DNA, 24 bp, Artificial Sequence
  Synthetic
ggttacacctttaacagctatggt

SEQ ID NO: 100 - protein, 8 aa, Artificial Sequence
  Synthetic
GYTFNSYG

SEQ ID NO: 101 - DNA, 24 bp, Artificial Sequence
  Synthetic
atcagctcccacaatggtaacagt

SEQ ID NO: 102 - protein, 8 aa, Artificial Sequence
  Synthetic
ISSHNGNS

SEQ ID NO: 103 - DNA, 45 bp, Artificial Sequence
  Synthetic
gcgagacactcgtataccaccagctggtacgggggttttgactat

SEQ ID NO: 104 - protein, 15 aa, Artificial Sequence
  Synthetic
ARHSYTTSWYGGFDY

SEQ ID NO: 105 - DNA, 321 bp, Artificial Sequence
  Synthetic
gacatccagatgacccagtctccatcttccgtgtctgcatctgtaggagacagagtcaccatcacttgtcgggcgagtcagggttttagcagctggttagcctggtatcagcagaaaccagggaaagcccctcagctcctgatctatgctgcatccagtttgcaaagtggggtcccatcaaggttcagcggcagtggatctgggtcagatttcactctcaccatcagcagcctgcagcctgaagattttgcaacttactattgtcaacaggctaacagtttccctctcactttcggcggagggaccaaggtggagatcaaa

SEQ ID NO: 106 - protein, 107 aa, Artificial Sequence
  Synthetic
DIQMTQSPSSVSASVGDRVTITCRASQGFSSWLAWYQQKPGKAPQLLIYAASSLQSGVPSRFSGSGSGSDFTLTISSLQPEDFATYYCQQANSFPLTFGGGTKVEIK

SEQ ID NO: 107 - DNA, 18 bp, Artificial Sequence
  Synthetic
cagggttttagcagctgg

SEQ ID NO: 108 - protein, 6 aa, Artificial Sequence
  Synthetic
QGFSSW

SEQ ID NO: 109 - DNA, 9 bp, Artificial Sequence
  Synthetic
gctgcatcc

SEQ ID NO: 110 - protein, 3 aa, Artificial Sequence
  Synthetic
AAS

SEQ ID NO: 111 - DNA, 27 bp, Artificial Sequence
  Synthetic
caacaggctaacagtttccctctcact

SEQ ID NO: 112 - protein, 9 aa, Artificial Sequence
  Synthetic
QQANSFPLT

SEQ ID NO: 113 - DNA, 366 bp, Artificial Sequence
  Synthetic
gaggtgcagctggtggagtccgggggaggcttggttcagccgggggggtccctgagactctcctgtgcagcctctggaatcaccttgagcagctatggcatgagctgggtccgccaggctccagggaagggactggagtgggtcgcatccatttttggtagtggtggtggcccatactacgcagactccgtgaagggccggttcaccatgtccagagacaattccaagaacacgctgtatttgcaaatgaacagcctgagagccgaggacacggccgtatattattgtgcgaaagatcgatacagtgggagctactacggaggttttgactactggggccggggaaccctggtcaccgtctcctca

SEQ ID NO: 114 - protein, 122 aa, Artificial Sequence
  Synthetic
EVQLVESGGGLVQPGGSLRLSCAASGITLSSYGMSWVRQAPGKGLEWVASIFGSGGGPYYADSVKGRFTMSRDNSKNTLYLQMNSLRAEDTAVYYCAKDRYSGSYYGGFDYWGRGTLVTVSS

SEQ ID NO: 115 - DNA, 24 bp, Artificial Sequence
  Synthetic
ggaatcaccttgagcagctatggc

SEQ ID NO: 116 - protein, 8 aa, Artificial Sequence
  Synthetic
GITLSSYG

SEQ ID NO: 117 - DNA, 24 bp, Artificial Sequence
  Synthetic
atttttggtagtggtggtggccca

SEQ ID NO: 118 - protein, 8 aa, Artificial Sequence
  Synthetic
IFGSGGGP

SEQ ID NO: 119 - DNA, 45 bp, Artificial Sequence
  Synthetic
gcgaaagatcgatacagtgggagctactacggaggttttgactac

SEQ ID NO: 120 - protein, 15 aa, Artificial Sequence
  Synthetic
AKDRYSGSYYGGFDY

SEQ ID NO: 121 - DNA, 321 bp, Artificial Sequence
  Synthetic
gacatccagatgacccagtctccatcttccgtgtctgcatctgtaggagacagagtcaccatcacttgtcgggcgagtcagggtattaccagctggttagcctggtatcagcagaaaccagggaaagcccctacactcctgatctatgctgcatccagtttgcaaactggggtcccatcaaggttcagcggcagtggatctgggacagatttcactctcaccatcagcagcctgcagcctgaacattttgcaacttactattgtcaacaggctaacagtttccctcctactttcggcggagggaccaaggtggagatcaaa

SEQ ID NO: 122 - protein, 107 aa, Artificial Sequence
  Synthetic
DIQMTQSPSSVSASVGDRVTITCRASQGITSWLAWYQQKPGKAPTLLIYAASSLQTGVPSRFSGSGSGTDFTLTISSLQPEHFATYYCQQANSFPPTFGGGTKVEIK

SEQ ID NO: 123 - DNA, 18 bp, Artificial Sequence
  Synthetic
cagggtattaccagctgg

SEQ ID NO: 124 - protein, 6 aa, Artificial Sequence
  Synthetic
QGITSW

SEQ ID NO: 125 - DNA, 9 bp, Artificial Sequence
  Synthetic
gctgcatcc

SEQ ID NO: 126 - protein, 3 aa, Artificial Sequence
  Synthetic
AAS

SEQ ID NO: 127 - DNA, 27 bp, Artificial Sequence
  Synthetic
caacaggctaacagtttccctcctact

SEQ ID NO: 128 - protein, 9 aa, Artificial Sequence
  Synthetic
QQANSFPPT

SEQ ID NO: 129 - DNA, 366 bp, Artificial Sequence
  Synthetic
gaggtgcagctggtggagtctgggggaggcttggtacagcctggggggtccctaagactctcctgtgcagcctctggattcacctttagcagttatgccttgacctgggtccgccaggctccagggaaggggctggagtgggtctcttttattagtggtagtggtggtaggccattctacgcagactccgtgaagggccggttcaccatctccagagacaattccaagaacatgctgtatctgcaaatgaacagcctgagagccgaggacacggccatatattactgtgcgaagtccctgtataccaccagctggtacggggggttcgactcctggggccagggaaccctggtcaccgtctcctca

SEQ ID NO: 130 - protein, 122 aa, Artificial Sequence
  Synthetic
EVQLVESGGGLVQPGGSLRLSCAASGFTFSSYALTWVRQAPGKGLEWVSFISGSGGRPFYADSVKGRFTISRDNSKNMLYLQMNSLRAEDTAIYYCAKSLYTTSWYGGFDSWGQGTLVTVSS

SEQ ID NO: 131 - DNA, 24 bp, Artificial Sequence
  Synthetic
ggattcacctttagcagttatgcc

SEQ ID NO: 132 - protein, 8 aa, Artificial Sequence
  Synthetic
GFTFSSYA

SEQ ID NO: 133 - DNA, 24 bp, Artificial Sequence
  Synthetic
attagtggtagtggtggtaggcca

SEQ ID NO: 134 - protein, 8 aa, Artificial Sequence
  Synthetic
ISGSGGRP

SEQ ID NO: 135 - DNA, 45 bp, Artificial Sequence
  Synthetic
gcgaagtccctgtataccaccagctggtacggggggttcgactcc

SEQ ID NO: 136 - protein, 15 aa, Artificial Sequence
  Synthetic
AKSLYTTSWYGGFDS

SEQ ID NO: 137 - DNA, 321 bp, Artificial Sequence
  Synthetic
gacatccagatgacccagtctccatcttccgtgtctgcatctgtaggagacagagtcaccatcacttgtcgggcgagtcagggtgtcgtcagctggttagcctggtatcagcagaaaccagggaaagcccctaagctcctgatctatgctgcatccagtttgcaaagtggggtcccatcaaggttcagcggcagtggatctgggacagatttcactctcaccatcagcagcctgcagcctgaagattttgcaacttattattgtcaacagtctaacagtttccctttcactctcggccctgggaccaaagtggatatcaaa

SEQ ID NO: 138 - protein, 107 aa, Artificial Sequence
  Synthetic
DIQMTQSPSSVSASVGDRVTITCRASQGVVSWLAWYQQKPGKAPKLLIYAASSLQSGVPSRFSGSGSGTDFTLTISSLQPEDFATYYCQQSNSFPFTLGPGTKVDIK

SEQ ID NO: 139 - DNA, 18 bp, Artificial Sequence
  Synthetic
cagggtgtcgtcagctgg

SEQ ID NO: 140 - protein, 6 aa, Artificial Sequence
  Synthetic
QGVVSW

SEQ ID NO: 141 - DNA, 9 bp, Artificial Sequence
  Synthetic
gctgcatcc

SEQ ID NO: 142 - protein, 3 aa, Artificial Sequence
  Synthetic
AAS

SEQ ID NO: 143 - DNA, 24 bp, Artificial Sequence
  Synthetic
caacagtctaacagtttccctttc

SEQ ID NO: 144 - protein, 8 aa, Artificial Sequence
  Synthetic
QQSNSFPF

SEQ ID NO: 145 - DNA, 366 bp, Artificial Sequence
  Synthetic
caggtgcagctggtgcagtctggggctgaagtgaagaagcctggggcctcagtgaaggtctcctgcaaggcttctggatacaccttcaccggccactatatgtactggatgcgacaggcccctggacaagggcttgagtggatgggatggatcaaccctaacagtggtggcacaaactatgcacagaagtttcaggacagggtcaccatgaccagggacacgtccatcagcacagcctacatggagctgagcaggctgagatctgacgacacggccgtgtattactgtgcgagagggagatatggcagtagctggtacggggggtttgagtactggggccagggaaccctggtcaccgtctcctca

SEQ ID NO: 146 - protein, 122 aa, Artificial Sequence
  Synthetic
QVQLVQSGAEVKKPGASVKVSCKASGYTFTGHYMYWMRQAPGQGLEWMGWINPNSGGTNYAQKFQDRVTMTRDTSISTAYMELSRLRSDDTAVYYCARGRYGSSWYGGFEYWGQGTLVTVSS

SEQ ID NO: 147 - DNA, 24 bp, Artificial Sequence
  Synthetic
ggatacaccttcaccggccactat

SEQ ID NO: 148 - protein, 8 aa, Artificial Sequence
  Synthetic
GYTFTGHY

SEQ ID NO: 149 - DNA, 24 bp, Artificial Sequence
  Synthetic
atcaaccctaacagtggtggcaca

SEQ ID NO: 150 - protein, 8 aa, Artificial Sequence
  Synthetic
INPNSGGT

SEQ ID NO: 151 - DNA, 45 bp, Artificial Sequence
  Synthetic
gcgagagggagatatggcagtagctggtacggggggtttgagtac

SEQ ID NO: 152 - protein, 15 aa, Artificial Sequence
  Synthetic
ARGRYGSSWYGGFEY

SEQ ID NO: 153 - DNA, 321 bp, Artificial Sequence
  Synthetic
gacatccagatgacccagtctccatcttccgtgtctgcatctgttggagacagagtcaccatcacttgtcgggcgagtcagggtattaccagctggttagcctggtatcagcagaaaccagggaaagcccctaacctcctgatctatgctgcagccagtttacaaagtggggtcccatcaaggttcagcggcagtggatctgggacggatttcactctcaccatcagcagcctgcagcctgaagactttacaacttactattgtcaacaggcttacagtctccctctcactttcggcggagggaccaaggtggagatcaaa

SEQ ID NO: 154 - protein, 107 aa, Artificial Sequence
  Synthetic
DIQMTQSPSSVSASVGDRVTITCRASQGITSWLAWYQQKPGKAPNLLIYAAASLQSGVPSRFSGSGSGTDFTLTISSLQPEDFTTYYCQQAYSLPLTFGGGTKVEIK

SEQ ID NO: 155 - DNA, 18 bp, Artificial Sequence
  Synthetic
cagggtattaccagctgg

SEQ ID NO: 156 - protein, 6 aa, Artificial Sequence
  Synthetic
QGITSW

SEQ ID NO: 157 - DNA, 9 bp, Artificial Sequence
  Synthetic
gctgcagcc

SEQ ID NO: 158 - protein, 3 aa, Artificial Sequence
  Synthetic
AAA

SEQ ID NO: 159 - DNA, 27 bp, Artificial Sequence
  Synthetic
caacaggcttacagtctccctctcact

SEQ ID NO: 160 - protein, 9 aa, Artificial Sequence
  Synthetic
QQAYSLPLT

SEQ ID NO: 161 - DNA, 366 bp, Artificial Sequence
  Synthetic
caggtgcagctggtggagtctgggggaggcgtggtccagcctgggaggtccctgagactctcctgtgcagcctctggattcaccttcagtagctatggcttgcactgggtccgccagtctccaggcaaggggctggaatgggtggcacttatatcatatgacggaagtaataaatactatgcagactccgtgaagggccgattcaccatctccagagacaattccaagaacacgctgtatctgcaaatgaacagcctgagacctgaggacacggctggatatttctgtgcgaaatccctatatacaaccagctggtacgggggctttgactattggggccagggaaccctggtcaccgtctcctca

SEQ ID NO: 162 - protein, 122 aa, Artificial Sequence
  Synthetic
QVQLVESGGGVVQPGRSLRLSCAASGFTFSSYGLHWVRQSPGKGLEWVALISYDGSNKYYADSVKGRFTISRDNSKNTLYLQMNSLRPEDTAGYFCAKSLYTTSWYGGFDYWGQGTLVTVSS

SEQ ID NO: 163 - DNA, 24 bp, Artificial Sequence
  Synthetic
ggattcaccttcagtagctatggc

SEQ ID NO: 164 - protein, 8 aa, Artificial Sequence
  Synthetic
GFTFSSYG

SEQ ID NO: 165 - DNA, 24 bp, Artificial Sequence
  Synthetic
atatcatatgacggaagtaataaa

SEQ ID NO: 166 - protein, 8 aa, Artificial Sequence
  Synthetic
ISYDGSNK

SEQ ID NO: 167 - DNA, 45 bp, Artificial Sequence
  Synthetic
gcgaaatccctatatacaaccagctggtacgggggctttgactat

SEQ ID NO: 168 - protein, 15 aa, Artificial Sequence
  Synthetic
AKSLYTTSWYGGFDY

SEQ ID NO: 169 - DNA, 321 bp, Artificial Sequence
  Synthetic
gacatccagatgacccagtctccatcttccgtgtctgcatctgtaggagacagagtcaccatcacttgtcgggcgagtcagggtattagaagctggttagcctggtatcagcaaaaaccagggaaagcccctaacctcctgatctatgctgcgtccagtttgcaaagtggggtcccatcaaggttcagcggcagtggatctgggacagatttcactctcaccatcagcagcctgcagcctgaagattttgcaacttactattgtcaacaggctaacagtttccctcccactttcggccctgggaccaaagtggatatcaaa

SEQ ID NO: 170 - protein, 107 aa, Artificial Sequence
  Synthetic
DIQMTQSPSSVSASVGDRVTITCRASQGIRSWLAWYQQKPGKAPNLLIYAASSLQSGVPSRFSGSGSGTDFTLTISSLQPEDFATYYCQQANSFPPTFGPGTKVDIK

SEQ ID NO: 171 - DNA, 18 bp, Artificial Sequence
  Synthetic
cagggtattagaagctgg

SEQ ID NO: 172 - protein, 6 aa, Artificial Sequence
  Synthetic
QGIRSW

SEQ ID NO: 173 - DNA, 9 bp, Artificial Sequence
  Synthetic
gctgcgtcc

SEQ ID NO: 174 - protein, 3 aa, Artificial Sequence
  Synthetic
AAS

SEQ ID NO: 175 - DNA, 27 bp, Artificial Sequence
  Synthetic
caacaggctaacagtttccctcccact

SEQ ID NO: 176 - protein, 9 aa, Artificial Sequence
  Synthetic
QQANSFPPT

SEQ ID NO: 177 - DNA, 366 bp, Artificial Sequence
  Synthetic
gaggtgcagctggtggagtctgggggaggcttggtacagcctggggggtccctgagactctcctgtgcagcctctgggttcaccttcagcaactatgccatgacctgggtccgccaggctccagggaaggggctggagtgggtctcaactatcagtggcagtggtgataacacatactacgcagactccgtgcagggccggttcaccatctccagaggccattccaagaacacgctgtatctgcaaatgaacagcctgagagccgaggacacggccgtatattactgtgcgaaacctacgtatagcagaagctggtacggtgcttttgatttctggggccaagggacaatggtcaccgtctcttca

SEQ ID NO: 178 - protein, 122 aa, Artificial Sequence
  Synthetic
EVQLVESGGGLVQPGGSLRLSCAASGFTFSNYAMTWVRQAPGKGLEWVSTISGSGDNTYYADSVQGRFTISRGHSKNTLYLQMNSLRAEDTAVYYCAKPTYSRSWYGAFDFWGQGTMVTVSS

SEQ ID NO: 179 - DNA, 24 bp, Artificial Sequence
  Synthetic
gggttcaccttcagcaactatgcc

SEQ ID NO: 180 - protein, 8 aa, Artificial Sequence
  Synthetic
GFTFSNYA

SEQ ID NO: 181 - DNA, 24 bp, Artificial Sequence
  Synthetic
atcagtggcagtggtgataacaca

SEQ ID NO: 182 - protein, 8 aa, Artificial Sequence
  Synthetic
ISGSGDNT

SEQ ID NO: 183 - DNA, 45 bp, Artificial Sequence
  Synthetic
gcgaaacctacgtatagcagaagctggtacggtgcttttgatttc

SEQ ID NO: 184 - protein, 15 aa, Artificial Sequence
  Synthetic
AKPTYSRSWYGAFDF

SEQ ID NO: 185 - DNA, 321 bp, Artificial Sequence
  Synthetic
gacatccagatgacccagtctccatcctccgtgtctgcatctgtaggagacagagtcaccatcacttgtcgggcgagtcagggtattagcagctggttagcctggtatcagcagaaaccggggaaagcccctcaactcctgatctatgctgcatccagattgcaaagtggggtcccatcaaggttctggggcagtggatctgggacagatttcactctcaccatcagcagcctgcagcctgaagattttgcaacttactattgtcaacaggctaacaatttcccattcactttcggccctgggaccaaagtggatatcaaa

SEQ ID NO: 186 - protein, 107 aa, Artificial Sequence
  Synthetic
DIQMTQSPSSVSASVGDRVTITCRASQGISSWLAWYQQKPGKAPQLLIYAASRLQSGVPSRFWGSGSGTDFTLTISSLQPEDFATYYCQQANNFPFTFGPGTKVDIK

SEQ ID NO: 187 - DNA, 18 bp, Artificial Sequence
  Synthetic
cagggtattagcagctgg

SEQ ID NO: 188 - protein, 6 aa, Artificial Sequence
  Synthetic
QGISSW

SEQ ID NO: 189 - DNA, 9 bp, Artificial Sequence
  Synthetic
gctgcatcc

SEQ ID NO: 190 - protein, 3 aa, Artificial Sequence
  Synthetic
AAS

SEQ ID NO: 191 - DNA, 27 bp, Artificial Sequence
  Synthetic
caacaggctaacaatttcccattcact

SEQ ID NO: 192 - protein, 9 aa, Artificial Sequence
  Synthetic
QQANNFPFT

SEQ ID NO: 193 - DNA, 366 bp, Artificial Sequence
  Synthetic
caggttcagctggtgcagtctggagctgaggtgaagaagcctggggcctcagtgaaggtctcctgcaaggcttctggttacacctttaccagttatggtatcagctgggtgcgacaggcccctggacaaggccttgagtggatgggatggatccgcgcttacaatggttacacaaactatgcacagaagtttcagggcagagtcaccatgaccacagacacatccacgaacaccgcctacatggagctgaggaccctgaattctgacgatacggccgtttattactgtgcgagagatcgatatagtgggagcttccacggtaactttgactactggggccagggaaccctggtcaccgtctcctca

SEQ ID NO: 194 - protein, 122 aa, Artificial Sequence
  Synthetic
QVQLVQSGAEVKKPGASVKVSCKASGYTFTSYGISWVRQAPGQGLEWMGWIRAYNGYTNYAQKFQGRVTMTTDTSTNTAYMELRTLNSDDTAVYYCARDRYSGSFHGNFDYWGQGTLVTVSS

SEQ ID NO: 195 - DNA, 24 bp, Artificial Sequence
  Synthetic
ggttacacctttaccagttatggt

SEQ ID NO: 196 - protein, 8 aa, Artificial Sequence
  Synthetic
GYTFTSYG

SEQ ID NO: 197 - DNA, 24 bp, Artificial Sequence
  Synthetic
atccgcgcttacaatggttacaca

SEQ ID NO: 198 - protein, 8 aa, Artificial Sequence
  Synthetic
IRAYNGYT

SEQ ID NO: 199 - DNA, 45 bp, Artificial Sequence
  Synthetic
gcgagagatcgatatagtgggagcttccacggtaactttgactac

SEQ ID NO: 200 - protein, 15 aa, Artificial Sequence
  Synthetic
ARDRYSGSFHGNFDY

SEQ ID NO: 201 - DNA, 321 bp, Artificial Sequence
  Synthetic
gacatccagatgacccagtctccatcttccgtgtctgcgtctgtaggagacagagtgaccatcacttgtcgggcgagtcagggtattttcagctggttagcctggtatcagcagaaaccagggaaagcccctaaggtcctaatctatgctgcatccaatttggaaagtggggtcccatcaaggttcagcggcagtggatctgggacagatttcactctcaccatcagcagcctgcagcctgaagattttgcaacttactattgtcaacaggctaacagtttaccgctcactttcggcggagggaccaaggtggagatcaaa

SEQ ID NO: 202 - protein, 107 aa, Artificial Sequence
  Synthetic
DIQMTQSPSSVSASVGDRVTITCRASQGIFSWLAWYQQKPGKAPKVLIYAASNLESGVPSRFSGSGSGTDFTLTISSLQPEDFATYYCQQANSLPLTFGGGTKVEIK

SEQ ID NO: 203 - DNA, 18 bp, Artificial Sequence
  Synthetic
cagggtattttcagctgg

SEQ ID NO: 204 - protein, 6 aa, Artificial Sequence
  Synthetic
QGIFSW

SEQ ID NO: 205 - DNA, 9 bp, Artificial Sequence
  Synthetic
gctgcatcc

SEQ ID NO: 206 - protein, 3 aa, Artificial Sequence
  Synthetic
AAS

SEQ ID NO: 207 - DNA, 27 bp, Artificial Sequence
  Synthetic
caacaggctaacagtttaccgctcact

SEQ ID NO: 208 - protein, 9 aa, Artificial Sequence
  Synthetic
QQANSLPLT

SEQ ID NO: 209 - DNA, 366 bp, Artificial Sequence
  Synthetic
gaggtgcagctggtggagtctgggggaggcttggtccagcctggggggtccctgagactctcctgtgcagcctctggattcaccttcagtacctattctatgcactgggtccgccaggctccagggaagggactggaatatgtttcaactattaataataatggggataccacatattatgcagactctgtgaagggcagattcaccatctccagagacaattccaagaacacgctgtatcttcaactgggcagcctgagacctgaggacatggctgtgtattactgtgcgagacagacgtataccagcagctggtacggggggttcgactcctggggccagggaaccctggtcaccgtctcctca

SEQ ID NO: 210 - protein, 122 aa, Artificial Sequence
  Synthetic
EVQLVESGGGLVQPGGSLRLSCAASGFTFSTYSMHWVRQAPGKGLEYVSTINNNGDTTYYADSVKGRFTISRDNSKNTLYLQLGSLRPEDMAVYYCARQTYTSSWYGGFDSWGQGTLVTVSS

SEQ ID NO: 211 - DNA, 24 bp, Artificial Sequence
  Synthetic
ggattcaccttcagtacctattct

SEQ ID NO: 212 - protein, 8 aa, Artificial Sequence
  Synthetic
GFTFSTYS

SEQ ID NO: 213 - DNA, 24 bp, Artificial Sequence
  Synthetic
attaataataatggggataccaca

SEQ ID NO: 214 - protein, 8 aa, Artificial Sequence
  Synthetic
INNNGDTT

SEQ ID NO: 215 - DNA, 45 bp, Artificial Sequence
  Synthetic
gcgagacagacgtataccagcagctggtacggggggttcgactcc

SEQ ID NO: 216 - protein, 15 aa, Artificial Sequence
  Synthetic
ARQTYTSSWYGGFDS

SEQ ID NO: 217 - DNA, 321 bp, Artificial Sequence
  Synthetic
gacatccagatgacccagtctccatcttccgtgtctgcatctgtaggcgacagagtcaccatcacttgtcgggcgagtcagggtattaccagctggttagcctggtatcagcagaaaccagggaaagcccctaaactcctgatctatgctgcatccaatttgcaaagtggggtcccatcaaggttcagcggcagtggatctgggacagatttcactctcaccatcaccagcctgcagcctgaggattttgcaacttactattgtcaacaggctaacagtctcccattcactttcggccctgggaccaaagtggatatcaaa

SEQ ID NO: 218 - protein, 107 aa, Artificial Sequence
  Synthetic
DIQMTQSPSSVSASVGDRVTITCRASQGITSWLAWYQQKPGKAPKLLIYAASNLQSGVPSRFSGSGSGTDFTLTITSLQPEDFATYYCQQANSLPFTFGPGTKVDIK

SEQ ID NO: 219 - DNA, 18 bp, Artificial Sequence
  Synthetic
cagggtattaccagctgg

SEQ ID NO: 220 - protein, 6 aa, Artificial Sequence
  Synthetic
QGITSW

SEQ ID NO: 221 - DNA, 9 bp, Artificial Sequence
  Synthetic
gctgcatcc

SEQ ID NO: 222 - protein, 3 aa, Artificial Sequence
  Synthetic
AAS

SEQ ID NO: 223 - DNA, 27 bp, Artificial Sequence
  Synthetic
caacaggctaacagtctcccattcact

SEQ ID NO: 224 - protein, 9 aa, Artificial Sequence
  Synthetic
QQANSLPFT

SEQ ID NO: 225 - DNA, 366 bp, Artificial Sequence
  Synthetic
gaggtgcagctggtggagtctgggggaggcttggtacagcctggggggtccctgagactctcctgtgcagcctctggattcacccttagcagctatgccatgagctgggtccgccaggctccagggaaggggctggagtgggtctcagctattagtggtagtggtggcagcacatactacgcagactccgtgaagggccggttcaccatctccagagacaattccaagaactcgctgtatctgcaattgaacagcctgagagccgaggacacggccgtatattactgtgcgaagacgctgtatactaccagctggtacgggggcttccagcactggggccagggcaccctggtcactgtctcctca

SEQ ID NO: 226 - protein, 122 aa, Artificial Sequence
  Synthetic
EVQLVESGGGLVQPGGSLRLSCAASGFTLSSYAMSWVRQAPGKGLEWVSAISGSGGSTYYADSVKGRFTISRDNSKNSLYLQLNSLRAEDTAVYYCAKTLYTTSWYGGFQHWGQGTLVTVSS

SEQ ID NO: 227 - DNA, 24 bp, Artificial Sequence
  Synthetic
ggattcacccttagcagctatgcc

SEQ ID NO: 228 - protein, 8 aa, Artificial Sequence
  Synthetic
GFTLSSYA

SEQ ID NO: 229 - DNA, 24 bp, Artificial Sequence
  Synthetic
attagtggtagtggtggcagcaca

SEQ ID NO: 230 - protein, 8 aa, Artificial Sequence
  Synthetic
ISGSGGST

SEQ ID NO: 231 - DNA, 45 bp, Artificial Sequence
  Synthetic
gcgaagacgctgtatactaccagctggtacgggggcttccagcac

SEQ ID NO: 232 - protein, 15 aa, Artificial Sequence
  Synthetic
AKTLYTTSWYGGFQH

SEQ ID NO: 233 - DNA, 321 bp, Artificial Sequence
  Synthetic
gacatccagatgacccagtctccatcttccgtgtctgcatctataggagacagagtcaccatcacttgtcgggcgagtcagggaatcagcagttggttagcctggtatcagcagaaaccagggaaagtccctaagctcctgatctatgctgcgtcctctttgcaaagtgggttcccatcaaggttcagcggcagtggatctgggacagatttcactctcaccatcagtagcctgcagcccgaagattttgcaacttactattgtcaacagactcacagtttcccgtggacggtcggccaagggaccaaggtggaaatcaaa

SEQ ID NO: 234 - protein, 107 aa, Artificial Sequence
  Synthetic
DIQMTQSPSSVSASIGDRVTITCRASQGISSWLAWYQQKPGKVPKLLIYAASSLQSGFPSRFSGSGSGTDFTLTISSLQPEDFATYYCQQTHSFPWTVGQGTKVEIK

SEQ ID NO: 235 - DNA, 18 bp, Artificial Sequence
  Synthetic
cagggaatcagcagttgg

SEQ ID NO: 236 - protein, 6 aa, Artificial Sequence
  Synthetic
QGISSW

SEQ ID NO: 237 - DNA, 9 bp, Artificial Sequence
  Synthetic
gctgcgtcc

SEQ ID NO: 238 - protein, 3 aa, Artificial Sequence
  Synthetic
AAS

SEQ ID NO: 239 - DNA, 24 bp, Artificial Sequence
  Synthetic
caacagactcacagtttcccgtgg

SEQ ID NO: 240 - protein, 8 aa, Artificial Sequence
  Synthetic
QQTHSFPW

SEQ ID NO: 241 - DNA, 366 bp, Artificial Sequence
  Synthetic
gaggtgcagctggtggagtctgggggaggcttggtacagcctggggggtccctgagactctcctgtgcagcctctggattcacccttaggagctatttcatgacctgggtccgccaggttccagggaaggggctggagggggtctcagctattagtggcattagtggtggcacatactacacagactccgttaagggccggttcaccatctccagagacaattccaagaacacgctgtttctgcaaatgaacagcctgagagccgaggacacggccgtatatttctgtgcgagaacggtgtatagtagtagttactacgggggcttccagcactggggccagggcaccctggtcaccgtctcctca

SEQ ID NO: 242 - protein, 122 aa, Artificial Sequence
  Synthetic
EVQLVESGGGLVQPGGSLRLSCAASGFTLRSYFMTWVRQVPGKGLEGVSAISGISGGTYYTDSVKGRFTISRDNSKNTLFLQMNSLRAEDTAVYFCARTVYSSSYYGGFQHWGQGTLVTVSS

SEQ ID NO: 243 - DNA, 24 bp, Artificial Sequence
  Synthetic
ggattcacccttaggagctatttc

SEQ ID NO: 244 - protein, 8 aa, Artificial Sequence
  Synthetic
GFTLRSYF

SEQ ID NO: 245 - DNA, 24 bp, Artificial Sequence
  Synthetic
attagtggcattagtggtggcaca

SEQ ID NO: 246 - protein, 8 aa, Artificial Sequence
  Synthetic
ISGISGGT

SEQ ID NO: 247 - DNA, 45 bp, Artificial Sequence
  Synthetic
gcgagaacggtgtatagtagtagttactacgggggcttccagcac

SEQ ID NO: 248 - protein, 15 aa, Artificial Sequence
  Synthetic
ARTVYSSSYYGGFQH

SEQ ID NO: 249 - DNA, 321 bp, Artificial Sequence
  Synthetic
gacatccagatgacccagtctccatcttccgtgtctgtatctgtaggagacagagtcaccatcacttgtcgggcgagtcagggtattagcagttggttagcctggtatcagcagaaaccagggaaagcccctaagctcctgatctatgttgcatccagtttacaaagtggggtcccatcaaggttcagcggcagtggatctgggacagatttcactctcaccatcagcagcctgcagcctgaagattttgcaacttactattgtcaacagactaacagtttccctctcactttcggcggagggaccaaggtggagatcaaa

SEQ ID NO: 250 - protein, 107 aa, Artificial Sequence
  Synthetic
DIQMTQSPSSVSVSVGDRVTITCRASQGISSWLAWYQQKPGKAPKLLIYVASSLQSGVPSRFSGSGSGTDFTLTISSLQPEDFATYYCQQTNSFPLTFGGGTKVEIK

SEQ ID NO: 251 - DNA, 18 bp, Artificial Sequence
  Synthetic
cagggtattagcagttgg

SEQ ID NO: 252 - protein, 6 aa, Artificial Sequence
  Synthetic
QGISSW

SEQ ID NO: 253 - DNA, 9 bp, Artificial Sequence
  Synthetic
gttgcatcc

SEQ ID NO: 254 - protein, 3 aa, Artificial Sequence
  Synthetic
VAS

SEQ ID NO: 255 - DNA, 27 bp, Artificial Sequence
  Synthetic
caacagactaacagtttccctctcact

SEQ ID NO: 256 - protein, 9 aa, Artificial Sequence
  Synthetic
QQTNSFPLT

SEQ ID NO: 257 - DNA, 366 bp, Artificial Sequence
  Synthetic
gaggtgcagctggtggagtctgggggaggcttggtacagcctggggggtccctgagactctcctgtgcagcctctggattcacccttaggagttatgtcatgtactgggtccgccagggtccagggaaggggctggagggggtctcaggtattagtggcagtagtggtggcacatactacacagactccgtgaagggccggttcaccatctccagagacaattccaagaacacgctgtttctgcaaatgaacagcctgagagccgaggacacggccgtatatttctgtgcgagatcggtgtatagtaccacctggtacgggggcttccagcactggggccagggcaccctggtcaccgtctcctca

SEQ ID NO: 258 - protein, 122 aa, Artificial Sequence
  Synthetic
EVQLVESGGGLVQPGGSLRLSCAASGFTLRSYVMYWVRQGPGKGLEGVSGISGSSGGTYYTDSVKGRFTISRDNSKNTLFLQMNSLRAEDTAVYFCARSVYSTTWYGGFQHWGQGTLVTVSS

SEQ ID NO: 259 - DNA, 24 bp, Artificial Sequence
  Synthetic
ggattcacccttaggagttatgtc

SEQ ID NO: 260 - protein, 8 aa, Artificial Sequence
  Synthetic
GFTLRSYV

SEQ ID NO: 261 - DNA, 24 bp, Artificial Sequence
  Synthetic
attagtggcagtagtggtggcaca

SEQ ID NO: 262 - protein, 8 aa, Artificial Sequence
  Synthetic
ISGSSGGT

SEQ ID NO: 263 - DNA, 45 bp, Artificial Sequence
  Synthetic
gcgagatcggtgtatagtaccacctggtacgggggcttccagcac

SEQ ID NO: 264 - protein, 15 aa, Artificial Sequence
  Synthetic
ARSVYSTTWYGGFQH

SEQ ID NO: 265 - DNA, 321 bp, Artificial Sequence
  Synthetic
gacatccagatgacccagtctccatcttccgtgtctgtatctgtgggagacagagtcaccatcacttgtcgggcgagtcaggttattagcagttggttagcctggtatcagctgaaaccagggaaagcccctaaactcctgatctatgctgcatccagtttacaaagtggggtcccatcaaggttcagcggcagtggatctgggacagatttcactctcaccatcagcggcctgcagcctgaagattttgcagtttactattgtcaacagactaacagtttccctctcactttcggcggagggaccaaggtggagatcaaa

SEQ ID NO: 266 - protein, 107 aa, Artificial Sequence
  Synthetic
DIQMTQSPSSVSVSVGDRVTITCRASQVISSWLAWYQLKPGKAPKLLIYAASSLQSGVPSRFSGSGSGTDFTLTISGLQPEDFAVYYCQQTNSFPLTFGGGTKVEIK

SEQ ID NO: 267 - DNA, 18 bp, Artificial Sequence
  Synthetic
caggttattagcagttgg

SEQ ID NO: 268 - protein, 6 aa, Artificial Sequence
  Synthetic
QVISSW

SEQ ID NO: 269 - DNA, 9 bp, Artificial Sequence
  Synthetic
gctgcatcc

SEQ ID NO: 270 - protein, 3 aa, Artificial Sequence
  Synthetic
AAS

SEQ ID NO: 271 - DNA, 27 bp, Artificial Sequence
  Synthetic
caacagactaacagtttccctctcact

SEQ ID NO: 272 - protein, 9 aa, Artificial Sequence
  Synthetic
QQTNSFPLT

SEQ ID NO: 273 - DNA, 366 bp, Artificial Sequence
  Synthetic
gaggtgcagctggtggagtctgggggaaacttggaacagcctggggggtcccttagactctcctgtacagcctctggattcacctttagcagatctgccatgaactgggtccgccgggctccagggaaggggctggagtgggtctcaggaattagtggtagtggtggtcgaacatactacgcagactccgtgaagggccggttcaccatctccagagacaattccaagaatacgctatatctgcaaatgaacagcctgagcgccgaggacacggccgcatattactgtgcgaaagattcgtatactaccagttggtacggaggtatggacgtctggggccacgggaccacggtcaccgtctcctca

SEQ ID NO: 274 - protein, 122 aa, Artificial Sequence
  Synthetic
EVQLVESGGNLEQPGGSLRLSCTASGFTFSRSAMNWVRRAPGKGLEWVSGISGSGGRTYYADSVKGRFTISRDNSKNTLYLQMNSLSAEDTAAYYCAKDSYTTSWYGGMDVWGHGTTVTVSS

SEQ ID NO: 275 - DNA, 24 bp, Artificial Sequence
  Synthetic
ggattcacctttagcagatctgcc

SEQ ID NO: 276 - protein, 8 aa, Artificial Sequence
  Synthetic
GFTFSRSA

SEQ ID NO: 277 - DNA, 24 bp, Artificial Sequence
  Synthetic
attagtggtagtggtggtcgaaca

SEQ ID NO: 278 - protein, 8 aa, Artificial Sequence
  Synthetic
ISGSGGRT

SEQ ID NO: 279 - DNA, 45 bp, Artificial Sequence
  Synthetic
gcgaaagattcgtatactaccagttggtacggaggtatggacgtc

SEQ ID NO: 280 - protein, 15 aa, Artificial Sequence
  Synthetic
AKDSYTTSWYGGMDV

SEQ ID NO: 281 - DNA, 321 bp, Artificial Sequence
  Synthetic
gacatccagatgacccagtctccatcttccgtgtctgcatctgtaggagacagagtcaccatcacttgtcgggcgagtcagggtattttcagctggttagcctggtatcagcagaaaccaggaaaagcccctaagctcctgatctatgctgcttccagtttacaaagtggggtcccatcaagattcagcggcagtggatctgggacagatttcactctcaccatcagcagcctgcagcctgaggattttgcaatttactattgtcaacaggctaacagtgtcccgatcaccttcggccaagggacacgactggagattaaa

SEQ ID NO: 282 - protein, 107 aa, Artificial Sequence
  Synthetic
DIQMTQSPSSVSASVGDRVTITCRASQGIFSWLAWYQQKPGKAPKLLIYAASSLQSGVPSRFSGSGSGTDFTLTISSLQPEDFAIYYCQQANSVPITFGQGTRLEIK

SEQ ID NO: 283 - DNA, 18 bp, Artificial Sequence
  Synthetic
cagggtattttcagctgg

SEQ ID NO: 284 - protein, 6 aa, Artificial Sequence
  Synthetic
QGIFSW

SEQ ID NO: 285 - DNA, 9 bp, Artificial Sequence
  Synthetic
gctgcttcc

SEQ ID NO: 286 - protein, 3 aa, Artificial Sequence
  Synthetic
AAS

SEQ ID NO: 287 - DNA, 27 bp, Artificial Sequence
  Synthetic
caacaggctaacagtgtcccgatcacc

SEQ ID NO: 288 - protein, 9 aa, Artificial Sequence
  Synthetic
QQANSVPIT

SEQ ID NO: 289 - DNA, 366 bp, Artificial Sequence
  Synthetic
gaggtgcagctggtggagtctgggggaggcttggtacagcctggggggtccctgagactctcctgttcagcctctggattcacctttagcagctatgccatgaactgggtccgccaggctccagggaaggggctggagtgggtcaccgctattagtggcagtggtggtggcacatactacgcagactccgtgaagggccggttcaccatctccagagacaattccaagaactcgctgtttctgcaattgaacagcctgagagccgaggacacggccgtgtattactgtgcgaaacaaacgtataccagcagctggtacggtggctttgatatctggggccaggggacaatggtcaccgtctcttca

SEQ ID NO: 290 - protein, 122 aa, Artificial Sequence
  Synthetic
EVQLVESGGGLVQPGGSLRLSCSASGFTFSSYAMNWVRQAPGKGLEWVTAISGSGGGTYYADSVKGRFTISRDNSKNSLFLQLNSLRAEDTAVYYCAKQTYTSSWYGGFDIWGQGTMVTVSS

SEQ ID NO: 291 - DNA, 24 bp, Artificial Sequence
  Synthetic
ggattcacctttagcagctatgcc

SEQ ID NO: 292 - protein, 8 aa, Artificial Sequence
  Synthetic
GFTFSSYA

SEQ ID NO: 293 - DNA, 24 bp, Artificial Sequence
  Synthetic
attagtggcagtggtggtggcaca

SEQ ID NO: 294 - protein, 8 aa, Artificial Sequence
  Synthetic
ISGSGGGT

SEQ ID NO: 295 - DNA, 45 bp, Artificial Sequence
  Synthetic
gcgaaacaaacgtataccagcagctggtacggtggctttgatatc

SEQ ID NO: 296 - protein, 15 aa, Artificial Sequence
  Synthetic
AKQTYTSSWYGGFDI

SEQ ID NO: 297 - DNA, 321 bp, Artificial Sequence
  Synthetic
gacatccagatgacccagtcgccatcttccgtgtccgcgtctgtaggagacagagtcaccatcacttgtcgggcgagtcagggttttagttcctggttagcctggtatcagcagataccagggaaagcccccaagctcctgatctatgctgcatcaaggttgcaaagtggggtcccatccaggttccgcggcagtggatctgggacagatttcactctcaccatcagcagcctgcagcctgaggattttgcaacttactattgtcaacaggctaacagtttcccgctcactttcggcggagggaccaaggtggagatcaaa

SEQ ID NO: 298 - protein, 107 aa, Artificial Sequence
  Synthetic
DIQMTQSPSSVSASVGDRVTITCRASQGFSSWLAWYQQIPGKAPKLLIYAASRLQSGVPSRFRGSGSGTDFTLTISSLQPEDFATYYCQQANSFPLTFGGGTKVEIK

SEQ ID NO: 299 - DNA, 18 bp, Artificial Sequence
  Synthetic
cagggttttagttcctgg

SEQ ID NO: 300 - protein, 6 aa, Artificial Sequence
  Synthetic
QGFSSW

SEQ ID NO: 301 - DNA, 9 bp, Artificial Sequence
  Synthetic
gctgcatca

SEQ ID NO: 302 - protein, 3 aa, Artificial Sequence
  Synthetic
AAS

SEQ ID NO: 303 - DNA, 27 bp, Artificial Sequence
  Synthetic
caacaggctaacagtttcccgctcact

SEQ ID NO: 304 - protein, 9 aa, Artificial Sequence
  Synthetic
QQANSFPLT

SEQ ID NO: 305 - protein, 167 aa, Artificial Sequence
  Synthetic
SITGISPITESLASLSTYNDQSITFALEDESYEIYVEDLKKDKKKDKVLLSYYESQHPSSESGDGVDGKMLMVTLSPTKDFWLQANNKEHSVELHKCEKPLPDQAFFVLHNRSFNCVSFECKTDPGVFIGVKDNHLALIKVDYSENLGSENILFKLSEILEHHHHHH

SEQ ID NO: 306 - protein, 167 aa, Artificial Sequence; identical to SEQ ID NO: 305
  Synthetic

SEQ ID NO: 307 - DNA, 354 bp, Artificial Sequence
  Synthetic
caggtcaccttgaaggagtctggtcctgtgctggtgaaacccacagagagcctcacgctgacctgctccgtctctggattctcactcagtaatgttagaatgggtgtgagctggatccgtcagtccccagggaaggccctggagtggcttgcacacattttttcgaatgacgaaaaatcctacaccacatctctgaagaccaggctcaccatctccaaggacacctccagaagccaggtggtccttaccatgaccgacatggaccctggggacacagccacatattactgtgcacggatacggaatttggcctttaattactggggccagggaaccctggtcaccgtctcctca

SEQ ID NO: 308 - protein, 118 aa, Artificial Sequence
  Synthetic
QVTLKESGPVLVKPTESLTLTCSVSGFSLSNVRMGVSWIRQSPGKALEWLAHIFSNDEKSYTTSLKTRLTISKDTSRSQVVLTMTDMDPGDTATYYCARIRNLAFNYWGQGTLVTVSS

SEQ ID NO: 309 - DNA, 30 bp, Artificial Sequence
  Synthetic
ggattctcactcagtaatgttagaatgggt

SEQ ID NO: 310 - protein, 10 aa, Artificial Sequence
  Synthetic
GFSLSNVRMG

SEQ ID NO: 311 - DNA, 21 bp, Artificial Sequence
  Synthetic
attttttcgaatgacgaaaaa

SEQ ID NO: 312 - protein, 7 aa, Artificial Sequence
  Synthetic
IFSNDEK

SEQ ID NO: 313 - DNA, 30 bp, Artificial Sequence
  Synthetic
gcacggatacggaatttggcctttaattac

SEQ ID NO: 314 - protein, 10 aa, Artificial Sequence
  Synthetic
ARIRNLAFNY

SEQ ID NO: 315 - DNA, 339 bp, Artificial Sequence
  Synthetic
gacttcgtgatgacccagtctccagactccctggctgtgtctctgggcgagagggccaccatcaactgcaagtccagccagagtgtgttacacaggtccagcaataagaactacttagcttggtatcagcagaagccaggacagcctcctaacctgctcatttactgggcatctacccgggaatccggggtccctgaccgattcagtggcagcgggtctgggacagatttcactctcaccatcagcagcctgcaggctgaagatgtggcagtttattactgtcagcaatattatggtactctatttactttcggccctgggaccaaagtggatatcaaa

SEQ ID NO: 316 - protein, 113 aa, Artificial Sequence
  Synthetic
DFVMTQSPDSLAVSLGERATINCKSSQSVLHRSSNKNYLAWYQQKPGQPPNLLIYWASTRESGVPDRFSGSGSGTDFTLTISSLQAEDVAVYYCQQYYGTLFTFGPGTKVDIK

SEQ ID NO: 317 - DNA, 36 bp, Artificial Sequence
  Synthetic
cagagtgtgttacacaggtccagcaataagaactac

SEQ ID NO: 318 - protein, 12 aa, Artificial Sequence
  Synthetic
QSVLHRSSNKNY

SEQ ID NO: 319 - DNA, 9 bp, Artificial Sequence
  Synthetic
tgggcatct

SEQ ID NO: 320 - protein, 3 aa, Artificial Sequence
  Synthetic
WAS

SEQ ID NO: 321 - DNA, 27 bp, Artificial Sequence
  Synthetic
cagcaatattatggtactctatttact

SEQ ID NO: 322 - protein, 9 aa, Artificial Sequence
  Synthetic
QQYYGTLFT

SEQ ID NO: 323 - protein, 338 aa, Artificial Sequence
  synthetic Amino acids 1-310: Human ST2 (K19-S328 of accession number NP_057316.3) Amino acids 311-338: Myc-Myc-hexahistidine tag
KFSKQSWGLENEALIVRCPRQGKPSYTVDWYYSQTNKSIPTQERNRVFASGQLLKFLPAAVADSGIYTCIVRSPTFNRTGYANVTIYKKQSDCNVPDYLMYSTVSGSEKNSKIYCPTIDLYNWTAPLEWFKNCQALQGSRYRAHKSFLVIDNVMTEDAGDYTCKFIHNENGANYSVTATRSFTVKDEQGFSLFPVIGAPAQNEIKEVEIGKNANLTCSACFGKGTQFLAAVLWQLNGTKITDFGEPRIQQEEGQNQSFSNGLACLDMVLRIADVKEEDLLLQYDCLALNLHGLRRHTVRLSRKNPIDHHSEQKLISEEDLGGEQKLISEEDLHHHHHH